European Patent Application EP 4 289 432 A1, published December 13, 2023. Title: Formulation for oral administration comprising triazine derivatives. Applicant: Shionogi & Co., Ltd. The sequence listing filed with the application follows.

SEQUENCE LISTING (2 sequences)

SEQ ID NO: 1 - protein, 14 aa, synthetic construct
  REGION 1..14: note = Substrate Peptide
KTSAVLQSGFRKME

SEQ ID NO: 2 - protein, 7 aa, synthetic construct
  REGION 1..7: note = Internal Standard Peptide
KTSAVLQ